European Patent Application EP 4 635 983 A1, published October 22, 2025. Title: A novel antibody binding specifically to NPTXR and use thereof. Applicant: Ymmonubio AG. The sequence listing filed with the application follows.

SEQUENCE LISTING (16 sequences)

SEQ ID NO: 1 - protein, 500 aa, Homo sapiens
  REGION 1..500: note = NPTXR
MKFLAVLLAAGMLAFLGAVICIIASVPLAASPARALPGGADNASVASGAAASPGPQRSLSALHGAGGSAGPPALPGAPAASAHPLPPGPLFSRFLCTPLAAACPSGAQQGDAAGAAPGEREELLLLQSTAEQLRQTALQQEARIRADQDTIRELTGKLGRCESGLPRGLQGAGPRRDTMADGPWDSPALILELEDAVRALRDRIDRLEQELPARVNLSAAPAPVSAVPTGLHSKMDQLEGQLLAQVLALEKERVALSHSSRRQRQEVEKELDVLQGRVAELEHGSSAYSPPDAFKISIPIRNNYMYARVRKALPELYAFTACMWLRSRSSGTGQGTPFSYSVPGQANEIVLLEAGHEPMELLINDKVAQLPLSLKDNGWHHICIAWTTRDGLWSAYQDGELQGSGENLAAWHPIKPHGILILGQEQDTLGGRFDATQAFVGDIAQFNLWDHALTPAQVLGIANCTAPLLGNVLPWEDKLVEAFGGATKAAFDVCKGRAKA

SEQ ID NO: 2 - protein, 15 aa, synthetic construct
  REGION 1..15: note = peptide fragment of NPTXR
GLPRGLQGAGPRRDT

SEQ ID NO: 3 - protein, 18 aa, synthetic construct
  REGION 1..18: note = peptide fragment of NPTXR
CESGLPRGLQGAGPRRDT

SEQ ID NO: 4 - protein, 5 aa, synthetic construct
  REGION 1..5: note = HCDR 1
NYGMN

SEQ ID NO: 5 - protein, 17 aa, synthetic construct
  REGION 1..17: note = HCDR 2
WINTDIGEPTYSQKFQG

SEQ ID NO: 6 - protein, 4 aa, synthetic construct
  REGION 1..4: note = HCDR 3
EMDV

SEQ ID NO: 7 - protein, 11 aa, synthetic construct
  REGION 1..11: note = LCDR 1
RASQSISDYLH

SEQ ID NO: 8 - protein, 7 aa, synthetic construct
  REGION 1..7: note = LCDR 2
YVSHSIS

SEQ ID NO: 9 - protein, 9 aa, synthetic construct
  REGION 1..9: note = LCDR 3
LNGHSFPFT

SEQ ID NO: 10 - protein, 113 aa, synthetic construct
  REGION 1..113: note = VH domain
QVQLVQSGAEVKKPGASVKVSCKASGYTFTNYGMNWVRQAPGQRLEWMGWINTDIGEPTYSQKFQGRVTITRDTSASTAYMELSSLRSEDTAVYYCAREMDVWGQGTTVTVSS

SEQ ID NO: 11 - protein, 107 aa, synthetic construct
  REGION 1..107: note = VL domain
DIQMTQSPSSLSASVGDRVTITCRASQSISDYLHWYQQKPGKAPKLLIKYVSHSISGVPSRFSGSGSGTDFTLTISSLQPEDFATYYCLNGHSFPFTFGGGTKVEIK

SEQ ID NO: 12 - DNA, 339 bp, synthetic construct
  misc_feature 1..339: note = encoding VH of SEQ ID NO 10
  source 1..339: mol_type = other DNA
caggtgcagctggtgcagtctggcgctgaggtgaagaagcctggcgcctctgtgaaggtgtcctgcaaggcctccggctataccttcaccaactacggaatgaactgggtcagacaagcccctggacagagactggagtggatggggtggatcaacaccgacatcggggagcccacctactcccagaagttccaggggcgggtcacaatcacccgggatacctccgcaagcaccgcttacatggagctgtcttctctgcgcagcgaggacaccgctgtctactactgcgctcgcgagatggatgtctggggacaggggacaacagtcaccgtcagcagc

SEQ ID NO: 13 - DNA, 321 bp, synthetic construct
  misc_feature 1..321: note = encoding VL of SEQ ID NO 11
  source 1..321: mol_type = other DNA
gacatccagatgacccagtctccctcttctctgtctgcctctgtgggcgatcgggtgaccatcacctgtcgggcttcccagtccatctccgactacctgcactggtaccagcagaagcctggcaaggccccaaagctgctcatcaagtacgtgtcccactccatctccggcgtgccatctagattctctggatctggatctggaaccgacttcaccctcaccatctcctccctccagcctgaggacttcgccacctactactgcctcaacgggcactctttccctttcaccttcggaggagggaccaaggtggagatcaag

SEQ ID NO: 14 - protein, 18 aa, synthetic construct
  REGION 1..18: note = peptide fragment of mouse NPTXR
CESGLPRGLQDAGPRRDT

SEQ ID NO: 15 - protein, 17 aa, synthetic construct
  REGION 1..17: note = HCDR2 of AB-parental
WINTDIGEPTYAEEFKG

SEQ ID NO: 16 - protein, 4 aa, synthetic construct
  REGION 1..4: note = HCDR 3 of AB-parental
EMDS